European Patent Application EP 4 494 655 A1, published January 22, 2025. Title: Combination of a multispecific molecule with an immune checkpoint inhibitor. Applicant: Daiichi Sankyo Company, Limited. Application JP. The sequence listing filed with the application follows.

SEQUENCE LISTING (71 sequences)

SEQ ID NO: 1 - protein, 8 aa, Rattus norvegicus
GFSIRSYD

SEQ ID NO: 2 - protein, 8 aa, Rattus norvegicus
ISYDGSQK

SEQ ID NO: 3 - protein, 13 aa, Rattus norvegicus
ARGSSGHYEAFDI

SEQ ID NO: 4 - protein, 8 aa, Rattus norvegicus
SSNIGNNY

SEQ ID NO: 5 - skipped

SEQ ID NO: 6 - protein, 12 aa, Rattus norvegicus
GTWDSSLSAPWV

SEQ ID NO: 7 - protein, 8 aa, Rattus norvegicus
GVTFNYYG

SEQ ID NO: 8 - protein, 8 aa, Rattus norvegicus
ITRSGGRI

SEQ ID NO: 9 - protein, 11 aa, Rattus norvegicus
TLDGRDGWVAY

SEQ ID NO: 10 - protein, 8 aa, Rattus norvegicus
TGNIGSNY

SEQ ID NO: 11 - skipped

SEQ ID NO: 12 - protein, 8 aa, Rattus norvegicus
QSYSSGFI

SEQ ID NO: 13 - protein, 120 aa, Rattus norvegicus
EVQLVESGGGVVQPGRSLTPSCSASGFSIRSYDIHWVRQAPGKGLEWVATISYDGSQKYFADSVKGRFTIFRDESENMVYLQMSGLRVEDTAVYHCARGSSGHYEAFDIWGQGTMVTVSS

SEQ ID NO: 14 - protein, 111 aa, Rattus norvegicus
QSVLTQPPSVSAAPGQKVTISCSGSSSNIGNNYVSWYQQLPGTAPKLLIYDNNKRPSGIPDRFSGSKSGTSATLGITGLQTGDEADYYCGTWDSSLSAPWVFGGGTKVTVL

SEQ ID NO: 15 - protein, 120 aa, synthetic construct; identical to SEQ ID NO: 13
  REGION 1..120: note = humanized

SEQ ID NO: 16 - protein, 111 aa, synthetic construct
  REGION 1..111: note = humanized
QSVLTQPPSVSAAPGQKVTISCSGSSSNIGNNYVSWYQRLPGTAPKLLIYDNNKRPSGIPDRFSGSKSGTSATLGITGLQTGDEADYYCGSWDSSLSAPWVFGGGTKVTVL

SEQ ID NO: 17 - protein, 292 aa, synthetic construct
  REGION 1..292: note = humanized
MKHLWFFLLLVAAPRWVLSGEVQLVESGGGVVQPGRSLTPSCSASGFSIRSYDIHWVRLAPGKGLEWVATISYDGSQKYFADSVKGRFTIFRDESENMVYLQMSGLRVEDTAVYHCARGSSGHYEAFDIWGQGTMVTVSSGGGGSGGGGSGGGGSQSVLTQPPSVSAAPGQKVTISCSGSSSNIGNNYVSWYQQLPGTAPKLLIYDNNKRPSGIPDRFSGSKSGTSATLGITGLQTGDEADYYCGTWDSSLSAPWVFGGGTKVTVLGAAAGAGGDYKDDDDKGAAAHHHHHH

SEQ ID NO: 18 - protein, 292 aa, synthetic construct
  REGION 1..292: note = humanized
MKHLWFFLLLVAAPRWVLSGEVQLVESGGGVVQPGRSLTPSCSASGFSIRSYDIHWVRQAPGKGLEWVATISYDGSQKYFADSVKGRFTIFRDESENMVYLQMSGLRVEDTAVYHCARGSSGHYEAFDIWGQGTMVTVSSGGGGSGGGGSGGGGSQSVLTQPPSVSAAPGQKVTISCSGSSSNIGNWYVSWYQQLPGTAPKLLIYDNNKRPSGIPDRFSGSKSGTSATLGITGLQTGDEADYYCGTWDSSLSAPWVFGGGTKVTVLGAAAGAGGDYKDDDDKGAAAHHHHHH

SEQ ID NO: 19 - protein, 292 aa, synthetic construct
  REGION 1..292: note = humanized
MKHLWFFLLLVAAPRWVLSGEVQLVESGGGVVQPGRSLTPSCSASGFSIRSYDIHWVRQAPGKGLEWVATISYDGSQKYFADSVKGRFTIFRDESENMVYLQMSGLRVEDTAVYHCARGSSGHYEAFDIWGQGTMVTVSSGGGGSGGGGSGGGGSQSVLTQPPSVSAAPGQKVTISCSGSSSNIGNNYVSWYQQLPGTAPKLLIYDNNKRPSGIPDRFSGSKSGTSATLGITGLQTGDEADYYCGSWDSSLSAPWVFGGGTKVTVLGAAAGAGGDYKDDDDKGAAAHHHHHH

SEQ ID NO: 20 - protein, 292 aa, synthetic construct
  REGION 1..292: note = humanized
MKHLWFFLLLVAAPRWVLSGEVQLVESGGGVVQPGRSLTPSCSASGFSIRSYDIHWVRLAPGKGLEWVATISYDGSQKYFADSVKGRFTIFRDESENMVYLQMSGLRVEDTAVYHCARGSSGHYEAFDIWGQGTMVTVSSGGGGSGGGGSGGGGSQSVLTQPPSVSAAPGQKVTISCSGSSSNIGNWYVSWYQQLPGTAPKLLIYDNNKRPSGIPDRFSGSKSGTSATLGITGLQTGDEADYYCGTWDSSLSAPWVFGGGTKVTVLGAAAGAGGDYKDDDDKGAAAHHHHHH

SEQ ID NO: 21 - protein, 292 aa, synthetic construct
  REGION 1..292: note = humanized
MKHLWFFLLLVAAPRWVLSGEVQLVESGGGVVQPGRSLTPSCSASGFSIRSYDIHWVRLAPGKGLEWVATISYDGSQKYFADSVKGRFTIFRDESENMVYLQMSGLRVEDTAVYHCARGSSGHYEAFDIWGQGTMVTVSSGGGGSGGGGSGGGGSQSVLTQPPSVSAAPGQKVTISCSGSSSNIGNWYVSWYQRLPGTAPKLLIYDNNKRPSGIPDRFSGSKSGTSATLGITGLQTGDEADYYCGTWDSSLSAPWVFGGGTKVTVLGAAAGAGGDYKDDDDKGAAAHHHHHH

SEQ ID NO: 22 - protein, 292 aa, synthetic construct
  REGION 1..292: note = humanized
MKHLWFFLLLVAAPRWVLSGEVQLVESGGGVVQPGRSLTPSCSASGFSIRSYDIHWVRLAPGKGLEWVATISYDGSQKYFADSVKGRFTIFRDESENMVYLQMSGLRVEDTAVYHCARGSSGHYEAFDIWGQGTMVTVSSGGGGSGGGGSGGGGSQSVLTQPPSVSAAPGQKVTISCSGSSSNIGNWKVSWYQQLPGTAPKLLIYDNNKRPSGIPDRFSGSKSGTSATLGITGLQTGDEADYYCGTWDSSLSAPWVFGGGTKVTVLGAAAGAGGDYKDDDDKGAAAHHHHHH

SEQ ID NO: 23 - protein, 111 aa, synthetic construct
  REGION 1..111: note = humanized
QSVLTQPPSASGTPGQRVTISCSGSSSNIGNWYVSWYQQLPGTAPKLLIYDNNKRPSGVPDRFSGSKSGTSASLAISGLQSEDEADYYCGTWDSSLSAPWVFGGGTKLTVL

SEQ ID NO: 24 - protein, 292 aa, synthetic construct
  REGION 1..292: note = humanized
MKHLWFFLLLVAAPRWVLSGEVQLVESGGGLVQPGGSLRLSCAASGFSIRSYDIHWVRLAPGKGLEWVATISYDGSQKYYADSVKGRFTISRDESKNTLYLQMNSLRAEDTAVYHCARGSSGHYEAFDIWGQGTLVTVSSGGGGSGGGGSGGGGSQSVLTQPPSVSAAPGQKVTISCSGSSSNIGNWYVSWYQQLPGTAPKLLIYDNNKRPSGIPDRFSGSKSGTSATLGITGLQTGDEADYYCGTWDSSLSAPWVFGGGTKVTVLGAAAGAGGDYKDDDDKGAAAHHHHHH

SEQ ID NO: 25 - protein, 292 aa, synthetic construct
  REGION 1..292: note = humanized
MKHLWFFLLLVAAPRWVLSGEVQLVESGGGLVQPGGSLRLSCAASGFSIRSYDIHWVRLAPGKGLEWVATISYDGSQKYYADSVKGRFTISRDESKNTLYLQMNSLRAEDTAVYHCARGSSGHYEAFDIWGQGTLVTVSSGGGGSGGGGSGGGGSQSVLTQPPSASGTPGQRVTISCSGSSSNIGNWYVSWYQQLPGTAPKLLIYDNNKRPSGVPDRFSGSKSGTSASLAISGLQSEDEADYYCGTWDSSLSAPWVFGGGTKLTVLGAAAGAGGDYKDDDDKGAAAHHHHHH

SEQ ID NO: 26 - protein, 292 aa, synthetic construct
  REGION 1..292: note = humanized
MKHLWFFLLLVAAPRWVLSGQVQLVESGGGVVQPGRSLRLSCAASGFSIRSYDMHWVRQAPGKGLEWVATISYDGSQKYYADSVKGRFTISRDNSKNTLYLQMSSLRAEDTAVYHCARGSSGHYEAFDIWGQGTLVTVSSGGGGSGGGGSGGGGSQSVLTQPPSVSAAPGQKVTISCSGSSSNIGNWYVSWYQQLPGTAPKLLIYDNNKRPSGIPDRFSGSKSGTSATLGITGLQTGDEADYYCGTWDSSLSAPWVFGGGTKVTVLGAAAGAGGDYKDDDDKGAAAHHHHHH

SEQ ID NO: 27 - protein, 292 aa, synthetic construct
  REGION 1..292: note = humanized
MKHLWFFLLLVAAPRWVLSGQVQLVESGGGVVQPGRSLRLSCAASGFSIRSYDMHWVRQAPGKGLEWVATISYDGSQKYYADSVKGRFTISRDNSKNTLYLQMSSLRAEDTAVYHCARGSSGHYEAFDIWGQGTLVTVSSGGGGSGGGGSGGGGSQSVLTQPPSASGTPGQRVTISCSGSSSNIGNWYVSWYQQLPGTAPKLLIYDNNKRPSGVPDRFSGSKSGTSASLAISGLQSEDEADYYCGTWDSSLSAPWVFGGGTKLTVLGAAAGAGGDYKDDDDKGAAAHHHHHH

SEQ ID NO: 28 - protein, 292 aa, synthetic construct
  REGION 1..292: note = humanized
MKHLWFFLLLVAAPRWVLSGEVQLVESGGGLVQPGGSLRLSCAASGFSIRSYDIHWVRQAPGKGLEWVATISYDGSQKYYADSVKGRFTISRDESKNTLYLQMNSLRAEDTAVYHCARGSSGHYEAFDIWGQGTLVTVSSGGGGSGGGGSGGGGSQSVLTQPPSVSAAPGQKVTISCSGSSSNIGNWYVSWYQQLPGTAPKLLIYDNNKRPSGIPDRFSGSKSGTSATLGITGLQTGDEADYYCGTWDSSLSAPWVFGGGTKVTVLGAAAGAGGDYKDDDDKGAAAHHHHHH

SEQ ID NO: 29 - protein, 292 aa, synthetic construct
  REGION 1..292: note = humanized
MKHLWFFLLLVAAPRWVLSGEVQLVESGGGLVQPGGSLRLSCAASGFSIRSYDIHWVRQAPGKGLEWVATISYDGSQKYYADSVKGRFTISRDESKNTLYLQMNSLRAEDTAVYHCARGSSGHYEAFDIWGQGTLVTVSSGGGGSGGGGSGGGGSQSVLTQPPSASGTPGQRVTISCSGSSSNIGNWYVSWYQQLPGTAPKLLIYDNNKRPSGVPDRFSGSKSGTSASLAISGLQSEDEADYYCGTWDSSLSAPWVFGGGTKLTVLGAAAGAGGDYKDDDDKGAAAHHHHHH

SEQ ID NO: 30 - protein, 292 aa, Rattus norvegicus
MKHLWFFLLLVAAPRWVLSGEVQLVESGGGVVQPGRSLTPSCSASGFSIRSYDIHWVRQAPGKGLEWVATISYDGSQKYFADSVKGRFTIFRDESENMVYLQMSGLRVEDTAVYHCARGSSGHYEAFDIWGQGTMVTVSSGGGGSGGGGSGGGGSQSVLTQPPSVSAAPGQKVTISCSGSSSNIGNNYVSWYQQLPGTAPKLLIYDNNKRPSGIPDRFSGSKSGTSATLGITGLQTGDEADYYCGTWDSSLSAPWVFGGGTKVTVLGAAAGAGGDYKDDDDKGAAAHHHHHH

SEQ ID NO: 31 - protein, 246 aa, Homo sapiens
MKHLWFFLLLVAAPRWVLSDKTHTCPPCPAPEAAGGPSVFLFPPKPKDTLMISRTPEVTCVVVSVSHEDPEVKFNWYVDGVEVHNAKTKPREEQYNSTYRVVSVLTVLHQDWLNGKEYKCKVSNKALPAPIEKTISKAKGQPREPQVYVLPPSRDELTKNQVSLLCLVKGFYPSDIAVEWESNGQPENNYLTWPPVLDSDGSFFLYSKLTVDKSRWQQGNVFSCSVMHEALHNHYTQKSLSLSPGK

SEQ ID NO: 32 - protein, 745 aa, synthetic construct
  REGION 1..745: note = humaized
MKHLWFFLLLVAAPRWVLSGEVQLVESGGGVVQPGRSLTPSCSASGFSIRSYDIHWVRLAPGKGLEWVATISYDGSQKYFADSVKGRFTIFRDESENMVYLQMSGLRVEDTAVYHCARGSSGHYEAFDIWGQGTMVTVSSGGGGSGGGGSGGGGSQSVLTQPPSVSAAPGQKVTISCSGSSSNIGNWYVSWYQQLPGTAPKLLIYDNNKRPSGIPDRFSGSKSGTSATLGITGLQTGDEADYYCGTWDSSLSAPWVFGGGTKVTVLGGGGSEVQLVESGGGLVQPGGSLRLSCAASGVTFNYYGMSWIRQAPGKGLEWVASITRSGGRIYYPDSVKGRFTISRENTQKTLYLQMNSLRAEDTAVYYCTLDGRDGWVAYWGQGTLVTVSSGGGGSGGGGSGGGGSNFMLTQPSSVSGVPGQRVTISCTGNTGNIGSNYVNWYQQLPGTAPKLLIYRDDKRPSGVPDRFSGSKSGTSASLAITGFQAEDEADYYCQSYSSGFIFGGGTKLTVLAAEPKSSDKTHTCPPCPAPEAAGGPSVFLFPPKPKDTLMISRTPEVTCVVVSVSHEDPEVKFNWYVDGVEVHNAKTKPREEQYNSTYRVVSVLTVLHQDWLNGKEYKCKVSNKALPAPIEKTISKAKGQPREPQVYVYPPSRDELTKNQVSLTCLVKGFYPSDIAVEWESNGQPENNYKTTPPVLDSDGSFALVSKLTVDKSRWQQGNVFSCSVMHEALHNHYTQKSLSLSPGK

SEQ ID NO: 33 - protein, 745 aa, synthetic construct
  REGION 1..745: note = humanized
MKHLWFFLLLVAAPRWVLSGEVQLVESGGGVVQPGRSLTPSCSASGFSIRSYDIHWVRLAPGKGLEWVATISYDGSQKYFADSVKGRFTIFRDESENMVYLQMSGLRVEDTAVYHCARGSSGHYEAFDIWGQGTMVTVSSGGGGSGGGGSGGGGSQSVLTQPPSVSAAPGQKVTISCSGSSSNIGNWYVSWYQRLPGTAPKLLIYDNNKRPSGIPDRFSGSKSGTSATLGITGLQTGDEADYYCGTWDSSLSAPWVFGGGTKVTVLGGGGSEVQLVESGGGLVQPGGSLRLSCAASGVTFNYYGMSWIRQAPGKGLEWVASITRSGGRIYYPDSVKGRFTISRENTQKTLYLQMNSLRAEDTAVYYCTLDGRDGWVAYWGQGTLVTVSSGGGGSGGGGSGGGGSNFMLTQPSSVSGVPGQRVTISCTGNTGNIGSNYVNWYQQLPGTAPKLLIYRDDKRPSGVPDRFSGSKSGTSASLAITGFQAEDEADYYCQSYSSGFIFGGGTKLTVLAAEPKSSDKTHTCPPCPAPEAAGGPSVFLFPPKPKDTLMISRTPEVTCVVVSVSHEDPEVKFNWYVDGVEVHNAKTKPREEQYNSTYRVVSVLTVLHQDWLNGKEYKCKVSNKALPAPIEKTISKAKGQPREPQVYVYPPSRDELTKNQVSLTCLVKGFYPSDIAVEWESNGQPENNYKTTPPVLDSDGSFALVSKLTVDKSRWQQGNVFSCSVMHEALHNHYTQKSLSLSPGK

SEQ ID NO: 34 - protein, 745 aa, synthetic construct
  REGION 1..745: note = humanized
MKHLWFFLLLVAAPRWVLSGEVQLVESGGGVVQPGRSLTPSCSASGFSIRSYDIHWVRLAPGKGLEWVATISYDGSQKYFADSVKGRFTIFRDESENMVYLQMSGLRVEDTAVYHCARGSSGHYEAFDIWGQGTMVTVSSGGGGSGGGGSGGGGSQSVLTQPPSVSAAPGQKVTISCSGSSSNIGNNYVSWYQQLPGTAPKLLIYDNNKRPSGIPDRFSGSKSGTSATLGITGLQTGDEADYYCGTWDSSLSAPWVFGGGTKVTVLGGGGSEVQLVESGGGLVQPGGSLRLSCAASGVTFNYYGMSWIRQAPGKGLEWVASITRSGGRIYYPDSVKGRFTISRENTQKTLYLQMNSLRAEDTAVYYCTLDGRDGWVAYWGQGTLVTVSSGGGGSGGGGSGGGGSNFMLTQPSSVSGVPGQRVTISCTGNTGNIGSNYVNWYQQLPGTAPKLLIYRDDKRPSGVPDRFSGSKSGTSASLAITGFQAEDEADYYCQSYSSGFIFGGGTKLTVLAAEPKSSDKTHTCPPCPAPEAAGGPSVFLFPPKPKDTLMISRTPEVTCVVVSVSHEDPEVKFNWYVDGVEVHNAKTKPREEQYNSTYRVVSVLTVLHQDWLNGKEYKCKVSNKALPAPIEKTISKAKGQPREPQVYVYPPSRDELTKNQVSLTCLVKGFYPSDIAVEWESNGQPENNYKTTPPVLDSDGSFALVSKLTVDKSRWQQGNVFSCSVMHEALHNHYTQKSLSLSPGK

SEQ ID NO: 35 - protein, 745 aa, synthetic construct
  REGION 1..745: note = humanized
MKHLWFFLLLVAAPRWVLSGEVQLVESGGGVVQPGRSLTPSCSASGFSIRSYDIHWVRQAPGKGLEWVATISYDGSQKYFADSVKGRFTIFRDESENMVYLQMSGLRVEDTAVYHCARGSSGHYEAFDIWGQGTMVTVSSGGGGSGGGGSGGGGSQSVLTQPPSVSAAPGQKVTISCSGSSSNIGNWYVSWYQQLPGTAPKLLIYDNNKRPSGIPDRFSGSKSGTSATLGITGLQTGDEADYYCGTWDSSLSAPWVFGGGTKVTVLGGGGSEVQLVESGGGLVQPGGSLRLSCAASGVTFNYYGMSWIRQAPGKGLEWVASITRSGGRIYYPDSVKGRFTISRENTQKTLYLQMNSLRAEDTAVYYCTLDGRDGWVAYWGQGTLVTVSSGGGGSGGGGSGGGGSNFMLTQPSSVSGVPGQRVTISCTGNTGNIGSNYVNWYQQLPGTAPKLLIYRDDKRPSGVPDRFSGSKSGTSASLAITGFQAEDEADYYCQSYSSGFIFGGGTKLTVLAAEPKSSDKTHTCPPCPAPEAAGGPSVFLFPPKPKDTLMISRTPEVTCVVVSVSHEDPEVKFNWYVDGVEVHNAKTKPREEQYNSTYRVVSVLTVLHQDWLNGKEYKCKVSNKALPAPIEKTISKAKGQPREPQVYVYPPSRDELTKNQVSLTCLVKGFYPSDIAVEWESNGQPENNYKTTPPVLDSDGSFALVSKLTVDKSRWQQGNVFSCSVMHEALHNHYTQKSLSLSPGK

SEQ ID NO: 36 - protein, 745 aa, synthetic construct
  REGION 1..745: note = humanized
MKHLWFFLLLVAAPRWVLSGEVQLVESGGGVVQPGRSLTPSCSASGFSIRSYDIHWVRQAPGKGLEWVATISYDGSQKYFADSVKGRFTIFRDESENMVYLQMSGLRVEDTAVYHCARGSSGHYEAFDIWGQGTMVTVSSGGGGSGGGGSGGGGSQSVLTQPPSVSAAPGQKVTISCSGSSSNIGNNYVSWYQQLPGTAPKLLIYDNNKRPSGIPDRFSGSKSGTSATLGITGLQTGDEADYYCGSWDSSLSAPWVFGGGTKVTVLGGGGSEVQLVESGGGLVQPGGSLRLSCAASGVTFNYYGMSWIRQAPGKGLEWVASITRSGGRIYYPDSVKGRFTISRENTQKTLYLQMNSLRAEDTAVYYCTLDGRDGWVAYWGQGTLVTVSSGGGGSGGGGSGGGGSNFMLTQPSSVSGVPGQRVTISCTGNTGNIGSNYVNWYQQLPGTAPKLLIYRDDKRPSGVPDRFSGSKSGTSASLAITGFQAEDEADYYCQSYSSGFIFGGGTKLTVLAAEPKSSDKTHTCPPCPAPEAAGGPSVFLFPPKPKDTLMISRTPEVTCVVVSVSHEDPEVKFNWYVDGVEVHNAKTKPREEQYNSTYRVVSVLTVLHQDWLNGKEYKCKVSNKALPAPIEKTISKAKGQPREPQVYVYPPSRDELTKNQVSLTCLVKGFYPSDIAVEWESNGQPENNYKTTPPVLDSDGSFALVSKLTVDKSRWQQGNVFSCSVMHEALHNHYTQKSLSLSPGK

SEQ ID NO: 37 - protein, 745 aa, synthetic construct
  REGION 1..745: note = humanized
MKHLWFFLLLVAAPRWVLSGEVQLVESGGGVVQPGRSLTPSCSASGFSIRSYDIHWVRLAPGKGLEWVATISYDGSQKYFADSVKGRFTIFRDESENMVYLQMSGLRVEDTAVYHCARGSSGHYEAFDIWGQGTMVTVSSGGGGSGGGGSGGGGSQSVLTQPPSVSAAPGQKVTISCSGSSSNIGNWKVSWYQQLPGTAPKLLIYDNNKRPSGIPDRFSGSKSGTSATLGITGLQTGDEADYYCGTWDSSLSAPWVFGGGTKVTVLGGGGSEVQLVESGGGLVQPGGSLRLSCAASGVTFNYYGMSWIRQAPGKGLEWVASITRSGGRIYYPDSVKGRFTISRENTQKTLYLQMNSLRAEDTAVYYCTLDGRDGWVAYWGQGTLVTVSSGGGGSGGGGSGGGGSNFMLTQPSSVSGVPGQRVTISCTGNTGNIGSNYVNWYQQLPGTAPKLLIYRDDKRPSGVPDRFSGSKSGTSASLAITGFQAEDEADYYCQSYSSGFIFGGGTKLTVLAAEPKSSDKTHTCPPCPAPEAAGGPSVFLFPPKPKDTLMISRTPEVTCVVVSVSHEDPEVKFNWYVDGVEVHNAKTKPREEQYNSTYRVVSVLTVLHQDWLNGKEYKCKVSNKALPAPIEKTISKAKGQPREPQVYVYPPSRDELTKNQVSLTCLVKGFYPSDIAVEWESNGQPENNYKTTPPVLDSDGSFALVSKLTVDKSRWQQGNVFSCSVMHEALHNHYTQKSLSLSPGK

SEQ ID NO: 38 - protein, 745 aa, synthetic construct
  REGION 1..745: note = humanized
MKHLWFFLLLVAAPRWVLSGEVQLVESGGGLVQPGGSLRLSCAASGFSIRSYDIHWVRLAPGKGLEWVATISYDGSQKYYADSVKGRFTISRDESKNTLYLQMNSLRAEDTAVYHCARGSSGHYEAFDIWGQGTLVTVSSGGGGSGGGGSGGGGSQSVLTQPPSVSAAPGQKVTISCSGSSSNIGNWYVSWYQQLPGTAPKLLIYDNNKRPSGIPDRFSGSKSGTSATLGITGLQTGDEADYYCGTWDSSLSAPWVFGGGTKVTVLGGGGSEVQLVESGGGLVQPGGSLRLSCAASGVTFNYYGMSWIRQAPGKGLEWVASITRSGGRIYYPDSVKGRFTISRENTQKTLYLQMNSLRAEDTAVYYCTLDGRDGWVAYWGQGTLVTVSSGGGGSGGGGSGGGGSNFMLTQPSSVSGVPGQRVTISCTGNTGNIGSNYVNWYQQLPGTAPKLLIYRDDKRPSGVPDRFSGSKSGTSASLAITGFQAEDEADYYCQSYSSGFIFGGGTKLTVLAAEPKSSDKTHTCPPCPAPEAAGGPSVFLFPPKPKDTLMISRTPEVTCVVVSVSHEDPEVKFNWYVDGVEVHNAKTKPREEQYNSTYRVVSVLTVLHQDWLNGKEYKCKVSNKALPAPIEKTISKAKGQPREPQVYVYPPSRDELTKNQVSLTCLVKGFYPSDIAVEWESNGQPENNYKTTPPVLDSDGSFALVSKLTVDKSRWQQGNVFSCSVMHEALHNHYTQKSLSLSPGK

SEQ ID NO: 39 - protein, 745 aa, synthetic construct
  REGION 1..745: note = humanized
MKHLWFFLLLVAAPRWVLSGEVQLVESGGGLVQPGGSLRLSCAASGFSIRSYDIHWVRLAPGKGLEWVATISYDGSQKYYADSVKGRFTISRDESKNTLYLQMNSLRAEDTAVYHCARGSSGHYEAFDIWGQGTLVTVSSGGGGSGGGGSGGGGSQSVLTQPPSASGTPGQRVTISCSGSSSNIGNWYVSWYQQLPGTAPKLLIYDNNKRPSGVPDRFSGSKSGTSASLAISGLQSEDEADYYCGTWDSSLSAPWVFGGGTKLTVLGGGGSEVQLVESGGGLVQPGGSLRLSCAASGVTFNYYGMSWIRQAPGKGLEWVASITRSGGRIYYPDSVKGRFTISRENTQKTLYLQMNSLRAEDTAVYYCTLDGRDGWVAYWGQGTLVTVSSGGGGSGGGGSGGGGSNFMLTQPSSVSGVPGQRVTISCTGNTGNIGSNYVNWYQQLPGTAPKLLIYRDDKRPSGVPDRFSGSKSGTSASLAITGFQAEDEADYYCQSYSSGFIFGGGTKLTVLAAEPKSSDKTHTCPPCPAPEAAGGPSVFLFPPKPKDTLMISRTPEVTCVVVSVSHEDPEVKFNWYVDGVEVHNAKTKPREEQYNSTYRVVSVLTVLHQDWLNGKEYKCKVSNKALPAPIEKTISKAKGQPREPQVYVYPPSRDELTKNQVSLTCLVKGFYPSDIAVEWESNGQPENNYKTTPPVLDSDGSFALVSKLTVDKSRWQQGNVFSCSVMHEALHNHYTQKSLSLSPGK

SEQ ID NO: 40 - protein, 745 aa, synthetic construct
  REGION 1..745: note = humanized
MKHLWFFLLLVAAPRWVLSGQVQLVESGGGVVQPGRSLRLSCAASGFSIRSYDMHWVRQAPGKGLEWVATISYDGSQKYYADSVKGRFTISRDNSKNTLYLQMSSLRAEDTAVYHCARGSSGHYEAFDIWGQGTLVTVSSGGGGSGGGGSGGGGSQSVLTQPPSVSAAPGQKVTISCSGSSSNIGNWYVSWYQQLPGTAPKLLIYDNNKRPSGIPDRFSGSKSGTSATLGITGLQTGDEADYYCGTWDSSLSAPWVFGGGTKVTVLGGGGSEVQLVESGGGLVQPGGSLRLSCAASGVTFNYYGMSWIRQAPGKGLEWVASITRSGGRIYYPDSVKGRFTISRENTQKTLYLQMNSLRAEDTAVYYCTLDGRDGWVAYWGQGTLVTVSSGGGGSGGGGSGGGGSNFMLTQPSSVSGVPGQRVTISCTGNTGNIGSNYVNWYQQLPGTAPKLLIYRDDKRPSGVPDRFSGSKSGTSASLAITGFQAEDEADYYCQSYSSGFIFGGGTKLTVLAAEPKSSDKTHTCPPCPAPEAAGGPSVFLFPPKPKDTLMISRTPEVTCVVVSVSHEDPEVKFNWYVDGVEVHNAKTKPREEQYNSTYRVVSVLTVLHQDWLNGKEYKCKVSNKALPAPIEKTISKAKGQPREPQVYVYPPSRDELTKNQVSLTCLVKGFYPSDIAVEWESNGQPENNYKTTPPVLDSDGSFALVSKLTVDKSRWQQGNVFSCSVMHEALHNHYTQKSLSLSPGK

SEQ ID NO: 41 - protein, 745 aa, synthetic construct
  REGION 1..745: note = humanized
MKHLWFFLLLVAAPRWVLSGQVQLVESGGGVVQPGRSLRLSCAASGFSIRSYDMHWVRQAPGKGLEWVATISYDGSQKYYADSVKGRFTISRDNSKNTLYLQMSSLRAEDTAVYHCARGSSGHYEAFDIWGQGTLVTVSSGGGGSGGGGSGGGGSQSVLTQPPSASGTPGQRVTISCSGSSSNIGNWYVSWYQQLPGTAPKLLIYDNNKRPSGVPDRFSGSKSGTSASLAISGLQSEDEADYYCGTWDSSLSAPWVFGGGTKLTVLGGGGSEVQLVESGGGLVQPGGSLRLSCAASGVTFNYYGMSWIRQAPGKGLEWVASITRSGGRIYYPDSVKGRFTISRENTQKTLYLQMNSLRAEDTAVYYCTLDGRDGWVAYWGQGTLVTVSSGGGGSGGGGSGGGGSNFMLTQPSSVSGVPGQRVTISCTGNTGNIGSNYVNWYQQLPGTAPKLLIYRDDKRPSGVPDRFSGSKSGTSASLAITGFQAEDEADYYCQSYSSGFIFGGGTKLTVLAAEPKSSDKTHTCPPCPAPEAAGGPSVFLFPPKPKDTLMISRTPEVTCVVVSVSHEDPEVKFNWYVDGVEVHNAKTKPREEQYNSTYRVVSVLTVLHQDWLNGKEYKCKVSNKALPAPIEKTISKAKGQPREPQVYVYPPSRDELTKNQVSLTCLVKGFYPSDIAVEWESNGQPENNYKTTPPVLDSDGSFALVSKLTVDKSRWQQGNVFSCSVMHEALHNHYTQKSLSLSPGK

SEQ ID NO: 42 - protein, 745 aa, synthetic construct
  REGION 1..745: note = humanized
MKHLWFFLLLVAAPRWVLSGEVQLVESGGGLVQPGGSLRLSCAASGFSIRSYDIHWVRQAPGKGLEWVATISYDGSQKYYADSVKGRFTISRDESKNTLYLQMNSLRAEDTAVYHCARGSSGHYEAFDIWGQGTLVTVSSGGGGSGGGGSGGGGSQSVLTQPPSVSAAPGQKVTISCSGSSSNIGNWYVSWYQQLPGTAPKLLIYDNNKRPSGIPDRFSGSKSGTSATLGITGLQTGDEADYYCGTWDSSLSAPWVFGGGTKVTVLGGGGSEVQLVESGGGLVQPGGSLRLSCAASGVTFNYYGMSWIRQAPGKGLEWVASITRSGGRIYYPDSVKGRFTISRENTQKTLYLQMNSLRAEDTAVYYCTLDGRDGWVAYWGQGTLVTVSSGGGGSGGGGSGGGGSNFMLTQPSSVSGVPGQRVTISCTGNTGNIGSNYVNWYQQLPGTAPKLLIYRDDKRPSGVPDRFSGSKSGTSASLAITGFQAEDEADYYCQSYSSGFIFGGGTKLTVLAAEPKSSDKTHTCPPCPAPEAAGGPSVFLFPPKPKDTLMISRTPEVTCVVVSVSHEDPEVKFNWYVDGVEVHNAKTKPREEQYNSTYRVVSVLTVLHQDWLNGKEYKCKVSNKALPAPIEKTISKAKGQPREPQVYVYPPSRDELTKNQVSLTCLVKGFYPSDIAVEWESNGQPENNYKTTPPVLDSDGSFALVSKLTVDKSRWQQGNVFSCSVMHEALHNHYTQKSLSLSPGK

SEQ ID NO: 43 - protein, 745 aa, synthetic construct
  REGION 1..745: note = humanized
MKHLWFFLLLVAAPRWVLSGEVQLVESGGGLVQPGGSLRLSCAASGFSIRSYDIHWVRQAPGKGLEWVATISYDGSQKYYADSVKGRFTISRDESKNTLYLQMNSLRAEDTAVYHCARGSSGHYEAFDIWGQGTLVTVSSGGGGSGGGGSGGGGSQSVLTQPPSASGTPGQRVTISCSGSSSNIGNWYVSWYQQLPGTAPKLLIYDNNKRPSGVPDRFSGSKSGTSASLAISGLQSEDEADYYCGTWDSSLSAPWVFGGGTKLTVLGGGGSEVQLVESGGGLVQPGGSLRLSCAASGVTFNYYGMSWIRQAPGKGLEWVASITRSGGRIYYPDSVKGRFTISRENTQKTLYLQMNSLRAEDTAVYYCTLDGRDGWVAYWGQGTLVTVSSGGGGSGGGGSGGGGSNFMLTQPSSVSGVPGQRVTISCTGNTGNIGSNYVNWYQQLPGTAPKLLIYRDDKRPSGVPDRFSGSKSGTSASLAITGFQAEDEADYYCQSYSSGFIFGGGTKLTVLAAEPKSSDKTHTCPPCPAPEAAGGPSVFLFPPKPKDTLMISRTPEVTCVVVSVSHEDPEVKFNWYVDGVEVHNAKTKPREEQYNSTYRVVSVLTVLHQDWLNGKEYKCKVSNKALPAPIEKTISKAKGQPREPQVYVYPPSRDELTKNQVSLTCLVKGFYPSDIAVEWESNGQPENNYKTTPPVLDSDGSFALVSKLTVDKSRWQQGNVFSCSVMHEALHNHYTQKSLSLSPGK

SEQ ID NO: 44 - protein, 468 aa, synthetic construct
  REGION 1..468: note = humanized
MKHLWFFLLLVAAPRWVLSEVQLVESGGGVVQPGRSLTPSCSASGFSIRSYDIHWVRQAPGKGLEWVATISYDGSQKYFADSVKGRFTIFRDESENMVYLQMSGLRVEDTAVYHCARGSSGHYEAFDIWGQGTMVTVSSASTKGPSVFPLAPSSKSTSGGTAALGCLVKDYFPEPVTVSWNSGALTSGVHTFPAVLQSSGLYSLSSVVTVPSSSLGTQTYICNVNHKPSNTKVDKRVEPKSCDKTHTCPPCPAPEAAGGPSVFLFPPKPKDTLMISRTPEVTCVVVSVSHEDPEVKFNWYVDGVEVHNAKTKPREEQYNSTYRVVSVLTVLHQDWLNGKEYKCKVSNKALPAPIEKTISKAKGQPREPQVYVLPPSRDELTKNQVSLLCLVKGFYPSDIAVEWESNGQPENNYLTWPPVLDSDGSFFLYSKLTVDKSRWQQGNVFSCSVMHEALHNHYTQKSLSLSPG

SEQ ID NO: 45 - protein, 237 aa, synthetic construct
  REGION 1..237: note = humanized
MVLQTQVFISLLLWISGAYGQSVLTQPPSVSAAPGQKVTISCSGSSSNIGNNYVSWYQQLPGTAPKLLIYDNNKRPSGIPDRFSGSKSGTSATLGITGLQTGDEADYYCGTWDSSLSAPWVFGGGTKVTVLGQPKAAPSVTLFPPSSEELQANKATLVCLISDFYPGAVTVAWKADSSPVKAGVETTTPSKQSNNKYAASSYLSLTPEQWKSHRSYSCQVTHEGSTVEKTVAPTECS

SEQ ID NO: 46 - protein, 269 aa, synthetic construct
  REGION 1..269: note = humanized
GEVQLVESGGGLVQPGGSLRLSCAASGVTFNYYGMSWIRQAPGKGLEWVASITNSGGRIYYPDSVKGRFTISRENTQKTLYLQMNSLRAEDTAVYYCTLDGRDGWVAYWGQGTLVTVSSGGGGSGGGGSGGGGSNFMLTQPHSVSESPGKTVTISCKRNTGNIGSNYVNWYQQHEGSSPTTIIYRDDKRPDGVSDRFSGSIDRSSKSASLTISNLKTEDEADYFCQSYSSGFIFGGGTKLTVLGAAAGAGGDYKDDDDKGAAAHHHHHH

SEQ ID NO: 47 - protein, 267 aa, synthetic construct
  REGION 1..267: note = humanized
GEVQLVESGGGLVQPGGSLRLSCAASGVTFNYYGMSWIRQAPGKGLEWVASITNSGGRIYYPDSVKGRFTISRENTQKTLYLQMNSLRAEDTAVYYCTLDGRDGWVAYWGQGTLVTVSSGGGGSGGGGSGGGGSNFMLTQPSSVSGVPGQRVTISCTGNTGNIGSNYVNWYQQLPGTAPKLLIYRDDKRPSGVPDRFSGSKSGTSASLAITGFQAEDEADYYCQSYSSGFIFGGGTKLTVLGAAAGAGGDYKDDDDKGAAAHHHHHH

SEQ ID NO: 48 - protein, 267 aa, synthetic construct
  REGION 1..267: note = humanized
GEVQLVESGGGLVQPGGSLRLSCAASGVTFNYYGMSWIRQAPGKGLEWVASITRSGGRIYYPDSVKGRFTISRENTQKTLYLQMNSLRAEDTAVYYCTLDGRDGWVAYWGQGTLVTVSSGGGGSGGGGSGGGGSNFMLTQPSSVSGVPGQRVTISCTGNTGNIGSNYVNWYQQLPGTAPKLLIYRDDKRPSGVPDRFSGSKSGTSASLAITGFQAEDEADYYCQSYSSGFIFGGGTKLTVLGAAAGAGGDYKDDDDKGAAAHHHHHH

SEQ ID NO: 49 - protein, 269 aa, synthetic construct
  REGION 1..269: note = humanized
GEVQLVESGGGLVQPGGSLRLSCAASGVTFNYYGMSWIRQAPGKGLEWVASITRSGGRIYYPDSVKGRFTISRENTQKTLYLQMNSLRAEDTAVYYCTLDGRDGWVAYWGQGTLVTVSSGGGGSGGGGSGGGGSNFMLTQPHSVSESPGKTVTISCKRNTGNIGSNYVNWYQQHEGSSPTTIIYRNDKRPDGVSDRFSGSIDRSSKSASLTISNLKTEDEADYFCQSYSSGFIFGGGTKLTVLGAAAGAGGDYKDDDDKGAAAHHHHHH

SEQ ID NO: 50 - protein, 269 aa, synthetic construct
  REGION 1..269: note = humanized
GEVQLVESGGGLVQPGGSLRLSCAASGVTFNYYGMSWIRQAPGKGLEWVASITSSGGRIYYPDSVKGRFTISRENTQKTLYLQMNSLRAEDTAVYYCTLDGRDGWVAYWGQGTLVTVSSGGGGSGGGGSGGGGSNFMLTQPHSVSESPGKTVTISCKRNTGNIGSNYVNWYQQHEGSSPTTIIYRNDKRPDGVSDRFSGSIDRSSKSASLTISNLKTEDEADYFCQSYSSGFIFGGGTKLTVLGAAAGAGGDYKDDDDKGAAAHHHHHH

SEQ ID NO: 51 - protein, 269 aa, synthetic construct
  REGION 1..269: note = humanized
GEVQLVESGGGLVQPGGSLRLSCAASGVTFNYYGMSWIRQAPGKGLEWVASITRSGGRIYYPDSVKGRFTISRENTQKTLYLQMNSLRAEDTAVYYCTLDGRDGWVAYWGQGTLVTVSSGGGGSGGGGSGGGGSNFMLTQPHSVSESPGKTVTISCKRNTGNIGSNYVNWYQQHEGSSPTTIIYRDDKRPDGVSDRFSGSIDRSSKSASLTISNLKTEDEADYFCQSYSSGFIFGGGTKLTVLGAAAGAGGDYKDDDDKGAAAHHHHHH

SEQ ID NO: 52 - protein, 745 aa, synthetic construct
  REGION 1..745: note = humanized
MKHLWFFLLLVAAPRWVLSGEVQLVESGGGVVQPGRSLTPSCSASGFSIRSYDIHWVRQAPGKGLEWVATISYDGSQKYFADSVKGRFTIFRDESENMVYLQMSGLRVEDTAVYHCARGSSGHYEAFDIWGQGTMVTVSSGGGGSGGGGSGGGGSQSVLTQPPSVSAAPGQKVTISCSGSSSNIGNNYVSWYQQLPGTAPKLLIYDNNKRPSGIPDRFSGSKSGTSATLGITGLQTGDEADYYCGTWDSSLSAPWVFGGGTKVTVLGGGGSEVQLVESGGGLVQPGGSLRLSCAASGVTFNYYGMSWIRQAPGKGLEWVASITRSGGRIYYPDSVKGRFTISRENTQKTLYLQMNSLRAEDTAVYYCTLDGRDGWVAYWGQGTLVTVSSGGGGSGGGGSGGGGSNFMLTQPSSVSGVPGQRVTISCTGNTGNIGSNYVNWYQQLPGTAPKLLIYRDDKRPSGVPDRFSGSKSGTSASLAITGFQAEDEADYYCQSYSSGFIFGGGTKLTVLAAEPKSSDKTHTCPPCPAPEAAGGPSVFLFPPKPKDTLMISRTPEVTCVVVSVSHEDPEVKFNWYVDGVEVHNAKTKPREEQYNSTYRVVSVLTVLHQDWLNGKEYKCKVSNKALPAPIEKTISKAKGQPREPQVYVYPPSRDELTKNQVSLTCLVKGFYPSDIAVEWESNGQPENNYKTTPPVLDSDGSFALVSKLTVDKSRWQQGNVFSCSVMHEALHNHYTQKSLSLSPGK

SEQ ID NO: 53 - protein, 745 aa, synthetic construct
  REGION 1..745: note = humanized
MKHLWFFLLLVAAPRWVLSGEVQLVESGGGVVQPGRSLTPSCSASGFSIRSYDIHWVRQAPGKGLEWVATISYDGSQKYFADSVKGRFTIFRDESENMVYLQMSGLRVEDTAVYHCARGSSGHYEAFDIWGQGTMVTVSSGGGGSGGGGSGGGGSQSVLTQPPSVSAAPGQKVTISCSGSSSNIGNNYVSWYQRLPGTAPKLLIYDNNKRPSGIPDRFSGSKSGTSATLGITGLQTGDEADYYCGSWDSSLSAPWVFGGGTKVTVLGGGGSEVQLVESGGGLVQPGGSLRLSCAASGVTFNYYGMSWIRQAPGKGLEWVASITRSGGRIYYPDSVKGRFTISRENTQKTLYLQMNSLRAEDTAVYYCTLDGRDGWVAYWGQGTLVTVSSGGGGSGGGGSGGGGSNFMLTQPSSVSGVPGQRVTISCTGNTGNIGSNYVNWYQQLPGTAPKLLIYRDDKRPSGVPDRFSGSKSGTSASLAITGFQAEDEADYYCQSYSSGFIFGGGTKLTVLAAEPKSSDKTHTCPPCPAPEAAGGPSVFLFPPKPKDTLMISRTPEVTCVVVSVSHEDPEVKFNWYVDGVEVHNAKTKPREEQYNSTYRVVSVLTVLHQDWLNGKEYKCKVSNKALPAPIEKTISKAKGQPREPQVYVYPPSRDELTKNQVSLTCLVKGFYPSDIAVEWESNGQPENNYKTTPPVLDSDGSFALVSKLTVDKSRWQQGNVFSCSVMHEALHNHYTQKSLSLSPGK

SEQ ID NO: 54 - protein, 745 aa, synthetic construct
  REGION 1..745: note = humanized
MKHLWFFLLLVAAPRWVLSGEVQLVESGGGLVQPGGSLRLSCAASGFSIRSYDIHWVRQAPGKGLEWVATISYDGSQKYYADSVKGRFTISRDESKNTLYLQMNSLRAEDTAVYHCARGSSGHYEAFDIWGQGTLVTVSSGGGGSGGGGSGGGGSQSVLTQPPSASGTPGQRVTISCSGSSSNIGNWYVSWYQQLPGTAPKLLIYDNNKRPSGVPDRFSGSKSGTSASLAISGLQSEDEADYYCGTWDSSLSAPWVFGGGTKLTVLGGGGSEVQLVESGGGLVQPGGSLRLSCAASGVTFNYYGMSWIRQAPGKGLEWVASITRSGGRIYYPDSVKGRFTISRENTQKTLYLQMNSLRAEDTAVYYCTLDGRDGWVAYWGCGTLVTVSSGGGGSGGGGSGGGGSNFMLTQPSSVSGVPGQRVTISCTGNTGNIGSNYVNWYQQLPGTCPKLLIYRDDKRPSGVPDRFSGSKSGTSASLAITGFQAEDEADYYCQSYSSGFIFGGGTKLTVLAAEPKSSDKTHTCPPCPAPEAAGGPSVFLFPPKPKDTLMISRTPEVTCVVVSVSHEDPEVKFNWYVDGVEVHNAKTKPREEQYNSTYRVVSVLTVLHQDWLNGKEYKCKVSNKALPAPIEKTISKAKGQPREPQVYVYPPSRDELTKNQVSLTCLVKGFYPSDIAVEWESNGQPENNYKTTPPVLDSDGSFALVSKLTVDKSRWQQGNVFSCSVMHEALHNHYTQKSLSLSPGK

SEQ ID NO: 55 - protein, 750 aa, synthetic construct
  REGION 1..750: note = humanized
MKHLWFFLLLVAAPRWVLSGEVQLVESGGGLVQPGGSLRLSCAASGFSIRSYDIHWVRQAPGKGLEWVATISYDGSQKYYADSVKGRFTISRDESKNTLYLQMNSLRAEDTAVYHCARGSSGHYEAFDIWGQGTLVTVSSGGGGSGGGGSGGGGSGGGGSQSVLTQPPSASGTPGQRVTISCSGSSSNIGNWYVSWYQQLPGTAPKLLIYDNNKRPSGVPDRFSGSKSGTSASLAISGLQSEDEADYYCGTWDSSLSAPWVFGGGTKLTVLGGGGSEVQLVESGGGLVQPGGSLRLSCAASGVTFNYYGMSWIRQAPGKGLEWVASITRSGGRIYYPDSVKGRFTISRENTQKTLYLQMNSLRAEDTAVYYCTLDGRDGWVAYWGCGTLVTVSSGGGGSGGGGSGGGGSNFMLTQPSSVSGVPGQRVTISCTGNTGNIGSNYVNWYQQLPGTCPKLLIYRDDKRPSGVPDRFSGSKSGTSASLAITGFQAEDEADYYCQSYSSGFIFGGGTKLTVLAAEPKSSDKTHTCPPCPAPEAAGGPSVFLFPPKPKDTLMISRTPEVTCVVVSVSHEDPEVKFNWYVDGVEVHNAKTKPREEQYNSTYRVVSVLTVLHQDWLNGKEYKCKVSNKALPAPIEKTISKAKGQPREPQVYVYPPSRDELTKNQVSLTCLVKGFYPSDIAVEWESNGQPENNYKTTPPVLDSDGSFALVSKLTVDKSRWQQGNVFSCSVMHEALHNHYTQKSLSLSPGK

SEQ ID NO: 56 - protein, 750 aa, synthetic construct
  REGION 1..750: note = humanized
MKHLWFFLLLVAAPRWVLSGEVQLVESGGGLVQPGGSLRLSCAASGFSIRSYDIHWVRQAPGKGLEWVATISYDGSQKYYADSVKGRFTISRDESKNTLYLQMNSLRAEDTAVYHCARGSSGHYEAFDIWGQGTLVTVSSGGGGSGGGGSGGGGSGGGGSQSVLTQPPSASGTPGQRVTISCSGSSSNIGNWYVSWYQQLPGTAPKLLIYDNNKRPSGVPDRFSGSKSGTSASLAISGLQSEDEADYYCGTWDSSLSAPWVFGGGTKLTVLGGGGSEVQLVESGGGLVQPGGSLRLSCAASGVTFNYYGMSWIRQAPGKCLEWVASITRSGGRIYYPDSVKGRFTISRENTQKTLYLQMNSLRAEDTAVYYCTLDGRDGWVAYWGQGTLVTVSSGGGGSGGGGSGGGGSNFMLTQPSSVSGVPGQRVTISCTGNTGNIGSNYVNWYQQLPGTAPKLLIYRDDKRPSGVPDRFSGSKSGTSASLAITGFQAEDEADYYCQSYSSGFIFGCGTKLTVLAAEPKSSDKTHTCPPCPAPEAAGGPSVFLFPPKPKDTLMISRTPEVTCVVVSVSHEDPEVKFNWYVDGVEVHNAKTKPREEQYNSTYRVVSVLTVLHQDWLNGKEYKCKVSNKALPAPIEKTISKAKGQPREPQVYVYPPSRDELTKNQVSLTCLVKGFYPSDIAVEWESNGQPENNYKTTPPVLDSDGSFALVSKLTVDKSRWQQGNVFSCSVMHEALHNHYTQKSLSLSPGK

SEQ ID NO: 57 - protein, 724 aa, synthetic construct
  REGION 1..724: note = humanized
MKHLWFFLLLVAAPRWVLSGEVQLVESGGGLVQPGGSLRLSCAASGFSIRSYDIHWVRQAPGKGLEWVATISYDGSQKYYADSVKGRFTISRDESKNTLYLQMNSLRAEDTAVYHCARGSSGHYEAFDIWGQGTLVTVSSGGGGSGGGGSGGGGSGGGGSQSVLTQPPSASGTPGQRVTISCSGSSSNIGNWYVSWYQQLPGTAPKLLIYDNNKRPSGVPDRFSGSKSGTSASLAISGLQSEDEADYYCGTWDSSLSAPWVFGGGTKLTVLGGGGSEVQLVESGGGLVQPGGSLRLSCAASGVTFNYYGMSWIRQAPGKGLEWVASITRSGGRIYYPDSVKGRFTISRENTQKTLYLQMNSLRAEDTAVYYCTLDGRDGWVAYWGQGTLVTVSSASTKGPSVFPLAPSSKSTSGGTAALGCLVKDYFPEPVTVSWNSGALTSGVHTFPAVLQSSGLYSLSSVVTVPSSSLGTQTYICNVNHKPSNTKVDKRVEPKSCDKTHTCPPCPAPEAAGGPSVFLFPPKPKDTLMISRTPEVTCVVVSVSHEDPEVKFNWYVDGVEVHNAKTKPREEQYNSTYRVVSVLTVLHQDWLNGKEYKCKVSNKALPAPIEKTISKAKGQPREPQVYVYPPSRDELTKNQVSLTCLVKGFYPSDIAVEWESNGQPENNYKTTPPVLDSDGSFALVSKLTVDKSRWQQGNVFSCSVMHEALHNHYTQKSLSLSPGK

SEQ ID NO: 58 - protein, 233 aa, synthetic construct
  REGION 1..233: note = humanized
MVLQTQVFISLLLWISGAYGNFMLTQPSSVSGVPGQRVTISCTGNTGNIGSNYVNWYQQLPGTAPKLLIYRDDKRPSGVPDRFSGSKSGTSASLAITGFQAEDEADYYCQSYSSGFIFGGGTKLTVLGQPKAAPSVTLFPPSSEELQANKATLVCLISDFYPGAVTVAWKADSSPVKAGVETTTPSKQSNNKYAASSYLSLTPEQWKSHRSYSCQVTHEGSTVEKTVAPTECS

SEQ ID NO: 59 - protein, 297 aa, synthetic construct
  REGION 1..297: note = humanized
MKHLWFFLLLVAAPRWVLSGEVQLVESGGGLVQPGGSLRLSCAASGFSIRSYDIHWVRQAPGKGLEWVATISYDGSQKYYADSVKGRFTISRDESKNTLYLQMNSLRAEDTAVYHCARGSSGHYEAFDIWGQGTLVTVSSGGGGSGGGGSGGGGSGGGGSQSVLTQPPSASGTPGQRVTISCSGSSSNIGNWYVSWYQQLPGTAPKLLIYDNNKRPSGVPDRFSGSKSGTSASLAISGLQSEDEADYYCGTWDSSLSAPWVFGGGTKLTVLGAAAGAGGDYKDDDDKGAAAHHHHHH

SEQ ID NO: 60 - protein, 719 aa, synthetic construct
  REGION 1..719: note = humanized
MKHLWFFLLLVAAPRWVLSGEVQLVESGGGLVQPGGSLRLSCAASGFSIRSYDIHWVRQAPGKGLEWVATISYDGSQKYYADSVKGRFTISRDESKNTLYLQMNSLRAEDTAVYHCARGSSGHYEAFDIWGQGTLVTVSSGGGGSGGGGSGGGGSQSVLTQPPSASGTPGQRVTISCSGSSSNIGNWYVSWYQQLPGTAPKLLIYDNNKRPSGVPDRFSGSKSGTSASLAISGLQSEDEADYYCGTWDSSLSAPWVFGGGTKLTVLGGGGSEVQLVESGGGLVQPGGSLRLSCAASGVTFNYYGMSWIRQAPGKGLEWVASITRSGGRIYYPDSVKGRFTISRENTQKTLYLQMNSLRAEDTAVYYCTLDGRDGWVAYWGQGTLVTVSSASTKGPSVFPLAPSSKSTSGGTAALGCLVKDYFPEPVTVSWNSGALTSGVHTFPAVLQSSGLYSLSSVVTVPSSSLGTQTYICNVNHKPSNTKVDKRVEPKSCDKTHTCPPCPAPEAAGGPSVFLFPPKPKDTLMISRTPEVTCVVVSVSHEDPEVKFNWYVDGVEVHNAKTKPREEQYNSTYRVVSVLTVLHQDWLNGKEYKCKVSNKALPAPIEKTISKAKGQPREPQVYVYPPSRDELTKNQVSLTCLVKGFYPSDIAVEWESNGQPENNYKTTPPVLDSDGSFALVSKLTVDKSRWQQGNVFSCSVMHEALHNHYTQKSLSLSPGK

SEQ ID NO: 61 - protein, 719 aa, synthetic construct
  REGION 1..719: note = humanized
MKHLWFFLLLVAAPRWVLSGQVQLVESGGGVVQPGRSLRLSCAASGFSIRSYDMHWVRQAPGKGLEWVATISYDGSQKYYADSVKGRFTISRDNSKNTLYLQMSSLRAEDTAVYHCARGSSGHYEAFDIWGQGTLVTVSSGGGGSGGGGSGGGGSQSVLTQPPSVSAAPGQKVTISCSGSSSNIGNWYVSWYQQLPGTAPKLLIYDNNKRPSGIPDRFSGSKSGTSATLGITGLQTGDEADYYCGTWDSSLSAPWVFGGGTKVTVLGGGGSEVQLVESGGGLVQPGGSLRLSCAASGVTFNYYGMSWIRQAPGKGLEWVASITRSGGRIYYPDSVKGRFTISRENTQKTLYLQMNSLRAEDTAVYYCTLDGRDGWVAYWGQGTLVTVSSASTKGPSVFPLAPSSKSTSGGTAALGCLVKDYFPEPVTVSWNSGALTSGVHTFPAVLQSSGLYSLSSVVTVPSSSLGTQTYICNVNHKPSNTKVDKRVEPKSCDKTHTCPPCPAPEAAGGPSVFLFPPKPKDTLMISRTPEVTCVVVSVSHEDPEVKFNWYVDGVEVHNAKTKPREEQYNSTYRVVSVLTVLHQDWLNGKEYKCKVSNKALPAPIEKTISKAKGQPREPQVYVYPPSRDELTKNQVSLTCLVKGFYPSDIAVEWESNGQPENNYKTTPPVLDSDGSFALVSKLTVDKSRWQQGNVFSCSVMHEALHNHYTQKSLSLSPGK

SEQ ID NO: 62 - protein, 240 aa, synthetic construct
  REGION 1..240: note = humanized
EVQLVESGGGLVQPGGSLRLSCAASGVTFNYYGMSWIRQAPGKGLEWVASITRSGGRIYYPDSVKGRFTISRENTQKTLYLQMNSLRAEDTAVYYCTLDGRDGWVAYWGCGTLVTVSSGGGGSGGGGSGGGGSNFMLTQPSSVSGVPGQRVTISCTGNTGNIGSNYVNWYQQLPGTCPKLLIYRDDKRPSGVPDRFSGSKSGTSASLAITGFQAEDEADYYCQSYSSGFIFGGGTKLTVL

SEQ ID NO: 63 - protein, 240 aa, synthetic construct
  REGION 1..240: note = humanized
EVQLVESGGGLVQPGGSLRLSCAASGVTFNYYGMSWIRQAPGKCLEWVASITRSGGRIYYPDSVKGRFTISRENTQKTLYLQMNSLRAEDTAVYYCTLDGRDGWVAYWGQGTLVTVSSGGGGSGGGGSGGGGSNFMLTQPSSVSGVPGQRVTISCTGNTGNIGSNYVNWYQQLPGTAPKLLIYRDDKRPSGVPDRFSGSKSGTSASLAITGFQAEDEADYYCQSYSSGFIFGCGTKLTVL

SEQ ID NO: 64 - protein, 242 aa, synthetic construct
  REGION 1..242: note = humanized
EVQLVESGGGLVQPGGSLRLSCAASGVTFNYYGMSWIRQAPGKGLEWVASITSSGGRIYYPDSVKGRFTISRENTQKTLYLQMNSLRAEDTAVYYCTLDGRDGWVAYWGCGTLVTVSSGGGGSGGGGSGGGGSNFMLTQPHSVSESPGKTVTISCKRNTGNIGSNYVNWYQQHEGSCPTTIIYRNDKRPDGVSDRFSGSIDRSSKSASLTISNLKTEDEADYFCQSYSSGFIFGGGTKLTVL

SEQ ID NO: 65 - protein, 242 aa, synthetic construct
  REGION 1..242: note = humanized
EVQLVESGGGLVQPGGSLRLSCAASGVTFNYYGMSWIRQAPGKCLEWVASITSSGGRIYYPDSVKGRFTISRENTQKTLYLQMNSLRAEDTAVYYCTLDGRDGWVAYWGQGTLVTVSSGGGGSGGGGSGGGGSNFMLTQPHSVSESPGKTVTISCKRNTGNIGSNYVNWYQQHEGSSPTTIIYRNDKRPDGVSDRFSGSIDRSSKSASLTISNLKTEDEADYFCQSYSSGFIFGCGTKLTVL

SEQ ID NO: 66 - protein, 9 aa, Homo sapiens
SLLMWITQC

SEQ ID NO: 67 - protein, 290 aa, Homo sapiens
MSHSMRYFFTSVSRPGRGEPRFIAVGYVDDTQFVRFDSDAASQRMEPRAPWIEQEGPEYWDGETRKVKAHSQTHRVDLGTLRGYYNQSEAGSHTVQRMYGCDVGSDWRFLRGYHQYAYDGKDYIALKEDLRSWTAADMAAQTTKHKWEAAHVAEQLRAYLEGTCVEWLRRYLENGKETLQRTDAPKTHMTHHAVSDHEATLRCWALSFYPAEITLTWQRDGEDQTQDTELVETRPAGDGTFQKWAAVVVPSGQEQRYTCHVQHEGLPKPLTLRWEGLNDIFEAQKIEWHE

SEQ ID NO: 68 - protein, 100 aa, Homo sapiens [sequence omitted]

SEQ ID NO: 69 - protein, 120 aa, synthetic construct
  REGION 1..120: note = humanized
QVQLVESGGGVVQPGRSLRLSCAASGFSIRSYDMHWVRQAPGKGLEWVATISYDGSQKYYADSVKGRFTISRDNSKNTLYLQMSSLRAEDTAVYHCARGSSGHYEAFDIWGQGTLVTVSS

SEQ ID NO: 70 - protein, 120 aa, synthetic construct
  REGION 1..120: note = humanized
EVQLVESGGGLVQPGGSLRLSCAASGFSIRSYDIHWVRQAPGKGLEWVATISYDGSQKYYADSVKGRFTISRDESKNTLYLQMNSLRAEDTAVYHCARGSSGHYEAFDIWGQGTLVTVSS

SEQ ID NO: 71 - protein, 292 aa, synthetic construct
  REGION 1..292: note = humanized
MKHLWFFLLLVAAPRWVLSGEVQLVESGGGVVQPGRSLTPSCSASGFSIRSYDMHWVRQAPGKGLEWVATISYDGSQKYFADSVKGRFTIFRDESENMVYLQMSGLRVEDTAVYHCARGSSNHYEAFDIWGQGTMVTVSSGGGGSGGGGSGGGGSQSVLTQPPSVSAAPGQKVTISCSGSSSNIGNNYVSWYQRLPGTAPKLLIYDNNKRPSGIPDRFSGSKSGTSATLGITGLQTGDEADYYCGAWDSSLSAPWVFGGGTKVTVLGAAAGAGGDYKDDDDKGAAAHHHHHH